European Patent Application EP 4 484 560 A1, published January 1, 2025. Title: TOBACCO PLANT AND METHOD FOR MANUFACTURING SAME. Applicant: JAPAN TOBACCO INC. The sequence listing filed with the application follows.

SEQUENCE LISTING (14 sequences)

SEQ ID NO: 1 - protein, 524 aa, Nicotiana tabacum
MECIGARNFSTMAVFTCPRFKSLGRKRIMPRKKQPFWPIHMKVKCSGSDSCVVVKEDFADEEDYIKAGGSELVFVQMQQNKDMDLQSKLSDKLRQISSAGQTILDLVVIGCGPAGLALAAESAKLGLNVGLVGPDLPFTNNYGVWEDEFKDLGLQACIEHVWSDTIVYLDDADPILIGRAYGRVSRHLLHEELLKRCVEAGVLYLNSKVDRIVESTSGHSLVECEGDIVIPCRFVTVASGAASGKFLQYELGGPRVSVQTAYGVEVEVDNNPYDPSLMVFMDYRDYVRHDAQSLEAKYPTFLYAMPMTKTRVFFEETCLASKDAMPFDLLKKKLMLRLNTLGIKIKKIYEEEWSYIPVGGSLPNTEQKTLAFGAAASMVHPATGYSVVRSLSEAPKCASVLANILRQNHVKNMITSSSATSISTQAWNTLWPQERKRQRSFFLFGLALILQLDIEGIRSFFRAFFRVPKWMWQGFLGSSLSSADLMLFAFYMFIIAPNDMRKGLIRHLLSDPTGATMIRTYLTF

SEQ ID NO: 2 - protein, 524 aa, Nicotiana tabacum
MDCIGARNFATMAVFTCPRFKSLGRRRIMPRKKQPIWPIHMQVKCSGNESCVVVKEDFADEEDYIKAGGSELVFVQMQQNKDMDLQSKLSDKLRQISSAGQTILDLVVIGCGPAGLALAAESAKLGLNVGLVGPDLPFTNNYGVWEDEFKDLGLQACIEHVWRDTIVYLDDADPILIGRAYGRVSRHLLHEELLKRCVEAGVLYLNSKVDRIVESTSGHSLVECEGDIVIPCRFVTVASGAASGKFLQYELGGPRVSVQTAYGVEVEVDNNPYDPSLMVFMDYRDYVRHDAQSLEAKYPTFLYAMPMTKTRVFFEETCLASKDAMPFDLLKKKLMLRLNTLGVRIKQIYEEEWSYIPVGGSLPNTEQKTLAFGAAASMVHPATGYSVVRSLSEAPKCASVLANILRQNHVKNMLTSSSTTSISTQAWNTLWPQERKRQRSFFLFGLALILQLDIEGIRSFFRAFFRVPKWMWQGFLGSSLSSADLMLFAFYMFIIAPNDMRKGLIRHLLSDPTGATMIRTYLTF

SEQ ID NO: 3 - DNA, 1575 bp, Nicotiana tabacum
  source 1..1575: mol_type = genomic DNA
atggagtgtattggagctcgaaatttttctacaatggcggtttttacgtgtccgagattcaaatcattaggaagaaagagaattatgccaagaaaaaagcaaccattttggcctatacatatgaaagtgaagtgtagtggaagtgatagttgtgtagtggttaaagaagattttgctgatgaagaagattatataaaagctggtggttcagaacttgtttttgttcaaatgcagcagaataaagacatggatctacagtctaagctttctgataagttgcgacaaatatcatcagctggacaaactatactggatttagtggtcattggctgtggtcctgctggtcttgctcttgctgcggagtctgctaaactcgggttgaacgtggggctcgttggtcctgatcttcctttcacaaataactatggtgtctgggaagacgagttcaaagatcttgggcttcaagcatgcattgaacatgtttggagtgataccattgtatatcttgatgatgccgatccaattcttattggacgtgcttatggaagagttagtcgccatttactgcatgaggagttactcaaaaggtgtgtggaggcaggtgttttatatcttaactcgaaagtggataggatcgttgagtccacaagtggccacagtcttgtagagtgcgagggcgacattgtcattccttgcaggtttgtcactgttgcatctggagccgcctcagggaaattcttgcagtatgagttgggaggtcctcgggtttctgttcaaacagcttatggagtggaagttgaggtcgataacaatccgtatgatccaagcctgatggttttcatggattatagagactatgtcagacacgacgctcaatctttagaagctaaatatccaacatttctttatgccatgcccatgactaaaacaagagtctttttcgaggaaacttgtttggcttcaaaagatgcaatgccatttgatctattaaagaaaaaactgatgttacgattgaacacattgggcataaaaattaaaaaaatctacgaggaggaatggtcttacataccagttggtggatcgttgccaaatacagagcagaaaacacttgcgtttggcgctgctgctagcatggttcatccagctacaggttattcagttgtcagatcactgtccgaggcgccaaaatgcgcctccgtacttgcaaatattttaagacaaaatcatgtcaagaacatgattaccagttcaagtgccacaagtatctcaactcaagcttggaacaccctttggccacaagaacgaaaaaggcaacgatcgtttttcctatttggattggcactcatattgcagctggatattgaggggattaggtcatttttccgcgcattcttccgtgtaccaaaatggatgtggcaaggttttcttggctctagtctttcatcagcagacctcatgttatttgccttctacatgtttattattgcaccaaatgacatgagaaaaggcctaatcagacatctgttatctgatccaactggtgcaactatgataagaacttatcttacattttag

SEQ ID NO: 4 - DNA, 1575 bp, Nicotiana tabacum
  source 1..1575: mol_type = genomic DNA
atggattgtattggagctcgaaattttgctacaatggcggtttttacgtgtccgagattcaaatcattaggaagaaggagaattatgccaagaaaaaagcaaccaatttggcctatacatatgcaagtgaagtgtagtggaaatgagagttgtgtagtagttaaagaagattttgccgatgaagaggattatataaaagctggtggttcagaacttgtttttgttcaaatgcagcagaataaagacatggatctgcagtctaagctttctgataagttgcgacaaatatcatcagctggacaaactatactggatttggtggtcataggctgtggtcctgctggtcttgctcttgctgcggagtctgctaaactcggattgaacgttgggctcgttggtcctgatcttcctttcacaaataactatggtgtttgggaggatgagttcaaagatcttgggcttcaagcgtgcattgaacatgtttggagggataccatagtatatcttgacgatgccgatccaattcttatcggtcgtgcttatggaagagttagtcgccatttactgcacgaggagttactcaaaaggtgtgtggaggcaggtgttttatatcttaactcgaaagtggataggatcgttgagtccacaagtggccacagtcttgtagagtgcgagggcgacattgtcattccttgcaggtttgtcactgttgcatctggtgctgcctcagggaaattcttgcagtatgagttgggaggtcctcgggtttctgttcaaacagcttatggagtggaagttgaggtcgataacaatccgtatgatccaagcctgatggttttcatggattatagagactatgtcagacacgacgctcaatctttagaagctaaatatccaacatttctttatgccatgcccatgactaaaacaagagtctttttcgaggaaacttgtttggcttcaaaagatgcaatgccatttgatttgttaaagaaaaaactgatgttacgattgaacacactgggtgtaagaattaagcaaatctacgaggaggaatggtcatacataccagttggtggatctttaccaaataccgagcaaaaaacacttgcatttggtgctgctgctagcatggttcatccagctacaggttattcagttgtcagatcactgtccgaggcaccaaaatgcgcctccgtacttgctaatattttacgacaaaatcatgtcaagaacatgctaaccagttcaagtaccacaagtatctcaactcaagcttggaacaccctttggccacaagaacgaaaaaggcaacgatcgtttttcctatttggattggcactcatattgcagttggatattgaggggattaggtcatttttccgcgcattcttccgtgtgccaaaatggatgtggcaaggatttcttggctctagtctttcatcagcagacctcatgttatttgccttctacatgtttattattgcaccaaatgacatgagaaaaggcctaatcagacatttgttatctgatccaactggtgcaaccatgataagaacttatcttacattttag

SEQ ID NO: 5 - DNA, 6356 bp, Nicotiana tabacum
  source 1..6356: mol_type = genomic DNA
aatcattattcaatatattcttcttaaattatatttcaatttattattttataaattcaatttcataagttattatactttctttttagttttagtaaaaaaatatatagctcttgaagattttaaaaaaaatccgaccttttcttttcgaaagctattctcaagttcctttgagaagacacaaacatggtgtagactaaatatatagtttgttttaatatacaactacattttgtatttaattactaaaagacatggctctattgaatagattatgctaatattcatcatttgtacgaatttatattttttctttgatatttgtccgataactcaaacacattattcaacaatatttatacaatttttaaaaattgtatgcttattaatataggtacacacgcaaagcgcgtaccccaaaactagtacaagaaaatatgcctcttgttttttttaagttcctttcaaactttcctttttctaaaaaaataaaaagacttatttgacaatatttgggtttaaaaaatctaaaaactgaaaaaagaaaaatcagaaatttattcacatgtttgaaaacaacgccaatgttgatcaattttctagagaacttcaaagcaatcaaagtatcaaacacaatagaaaattaaaaaataattcaaaaaaaaaaaagcgtctcaacattttcggaacgaaataactgcagctaatcaaatccatccacgtgtcattattgtgaaatgacagttgaacacatcagcaaaaagcttccctccttcctatccatatcttcactctctgtccatccaaaaaaccagcaaagactcacaaaactccattttaattcagcttcaattcttgctaatatttcatgcattttcaattttcataaccccattaaaccaaaagaatgaatgaaaatctcaaattttgaaaaatcttgagaaaagaaaaataaaccagaggagtcaaagaaagactatatataaattggagctcaaacatggagtgtattggagctcgaaatttttctacaatggcggtttttacgtgtccgagattcaaatcattaggaagaaagagaattatgccaagaaaaaagcaaccattttggcctatacatatgaaagtgaagtgtagtggaagtgatagttgtgtagtggttaaagaagattttgctgatgaagaagattatataaaagctggtggttcagaacttgtttttgttcaaatgcagcagaataaagacatggatctacagtctaagctttctgataaggtgattttcttgatcccatatttaaaaggatttaacttgtatacattaaggggtcgtttggtttgaagacaagttatgtcaggatcagttatggtgtgattagttatagtgggattagttatgttgggattagttattatttcttattgactgtttggtatgttctattaatcctatgattgtcaaatataatgttttattcccagataacttatcctatgattactattccaacctctggtaggtataagttatcccgatactatttttaatcatgggataacttattccgagcttagtaaccaaataagggataaggcgctactaaatttttatcccatgattatttttgctaatctatcgtaccatgcgacccctagaagggaagttcggtacacaaagcatcccgcattaatattcacgcagggtttgggtaagggccgggtccgaagggatgtgatgtagatagcctacctaatacaagtattagtggctgcttccatagtttgaacctttggtcacacggagacaactttactgttgttgtaaggttatcctttaacttgtatacattgtcagtataaattttttaacaatatctatgtaatttaacctgttataacaggttaattgctttattttttaggtaatcagttccacttattgtaaatgtagttacctatagttatctttaggtaacttgatagtgtaaatattcttttacactttcagctaattaaagtcaaattctgtttaaaaaggaaacaaacttatagtgtacagtggtagtgtgacaaaatcttacactatcagtgtattttaccttatattcgcgattactaaactattccaaattaccacacattgaattccatgtgagttagagttatgcaatatgaaagaaatgaagaagctagaaaaactaccatactgcagcaactatgtctgcaatttattttaactcttatattgtagcaaactatattgctttgtccatcatactatctcagcttgcagttgcgacaaatatcatcagctggacaaactatactggatttagtggtcattggctgtggtcctgctggtcttgctcttgctgcggagtctgctaaactcgggttgaacgtggggctcgttggtcctgatcttcctttcacaaataactatggtgtctgggaagacgagttcaaaggtcgtaatccttatttatcttttatgaagagtccttttctctacataacctttcaagaaacagaacctcttgttctctggagcttaatttagacatatgcttatactttcctttttcagatcttgggcttcaagcatgcattgaacatgtttggagtgataccattgtatatcttgatgatgccgatccaattcttattggacgtgcttatggaagagttagtcgccatttactgcatgaggagttactcaaaaggttaaattcactgaacttgttccttatgtcatacgagttgttgatttattccttacaattgaggttgtaattcacattaatcttcttaggtgtgtggaggcaggtgttttatatcttaactcgaaagtggataggatcgttgagtccacaagtggccacagtcttgtagagtgcgagggcgacattgtcattccttgcaggtatagttggaccgctacatcaaattgtcactgttcacgttagaaacttaactgcatccttgttctgatgcttctaacttatgataacaggtttgtcactgttgcatctggagccgcctcagggaaattcttgcagtatgagttgggaggtcctcgggtttctgttcaaacagcttatggagtggaagttgaggtagagaaatatcatcaaacctcgagtaactcttgagggtttttcatgttatgcaccagaagactttagactgttacctgtagttatcatttacgagcttatatgaacaatttgttgcattattccttttatggcctatcctttcactgctcgtcttggagagtacgcattcaatttggcgattctgtttctattgtaaacttagaattggacttcctataaggttatgcacattcaagaaaaccgctatctgcatttcccaattactagcttggctgattttgcaattatatgatcattcttcttttcttttttcctatatattaggtcgataacaatccgtatgatccaagcctgatggttttcatggattatagagactatgtcagacacgacgctcaatctttagaagctaaatatccaacatttctttatgccatgcccatgactaaaacaagagtctttttcgaggttagtttttgatattatgcctcatactttactacttggctttgtgtgacagacaaaagtatctatctgcaggaaacttgtttggcttcaaaagatgcaatgccatttgatctattaaagaaaaaactgatgttacgattgaacacattgggcataaaaattaaaaaaatctacgaggaggtaatccactctacctttagttacgtgcaatttttgctagagaaaaaaaagggcaacccggtgcaaagcacccgctatgcgcgggtccggggaagggctggaccacaagggtctattgtacgcaaccttaccctgcatttctgcaagagactgtttccacggctcgaattcgtgacctcttggtcgcatggcagcaactttaccagttacgccaaggctccccgtgaacacactagagaatgactgaaaaatgactttaacaaaattttacgcaggaatggtcttacataccagttggtggatcgttgccaaatacagagcagaaaacacttgcgtttggcgctgctgctagcatggttcatccagctacaggtaataagagaagaaaatacattactattactgtgttctttaaatgcaatgcttctgaaacttcctctacttcataaacaggttattcagttgtcagatcactgtccgaggcgccaaaatgcgcctccgtacttgcaaatattttaagacaaaatcatgtcaagaacatgattaccagttcaagtgccacaagtatctcaactcaaggtacttgttatccaattatactagtttttgactgcattggtagtgtcctgacctatatggactcagcaagttgctcatattttcttcagcttggaacaccctttggccacaagaacgaaaaaggcaacgatcgtttttcctatttggattggcactcatattgcagctggatattgaggggattaggtcatttttccgcgcattcttccgtgtaccaaaatggtatggtttgatcttgctccatcaccccgttatcttcgatcatgtggcatcgttttccaaatcagtttaacttctatacgctgacaatataaagaatttttaaactacaagatgaccaaaaaaaaactacgtgtaacggtttgtaataagtgagtcagtaacgcacaaaataaggcagggcaacatgatacaacaagttaagatacactaataccaacaacaacaacaactataccctctgtaccaaacaagttggagcggctatcagaggcggagctagagtgccccgaacgggttcggccgaacccagtagctttggttcaaaccctgtatttgtctctaaaaaattcattgaatatatataaattattaaattagaatccaatagcttaaaacgattagaatttcgaacccataaacttgaaatcctgactacctctggcgactgtatgaatcctcaatgactatccatgtaaattcttctcatgtcaacattatacgaaacaaaaatcaaaacgaaaagtacgtacaagttttctatgtttccaactgacataagaatcccaatagtctaaattctttagagtgtcagtgcatataatgagaagtgtacttattgcaggatgtggcaaggttttcttggctctagtctttcatcagcagacctcatgttatttgccttctacatgtttattattgcaccaaatgacatgagaaaaggcctaatcagacatctgttatctgatccaactggtgcaactatgataagaacttatcttacattttagagtagattcagaggagaaatcactgccttttgtatataacatttcactagattatattaatatgctcaaataaatgacaggaattcaatttttgtatctacttctttgtccaaatgtattgatccattgaactctattagcttcaataaatgaatgatgattttgctgataattgcttcgaataaatgagttatgatccttttagatatactactcgttactcccactcatacataatacatttctacgtgcttgacccataaaaagaaaaagaatcaaatacattacaaataatatgaatcgtctcatcggaaagaatcaatctttcttatgagacgatatattatttgtaatagaagagcttttgactataactatatcgccctacctttgacttgtttttttcacctaatctcttaaactgaaaatagccggcagatgtataatatatgtataattcatgaataatatatatatatatatgtgtataattaatatataatatatgtatatcagctaaaaaaagtaaacactaaatctggccggctacttgtgtaacaatccttttttttgtttctcatccagtgtccagtacccgcattggggtctggctaaatttggatttgcaccggaaagtaccatattgagggtaaagcgctccctaacaaaggcggcttcataaccaaggttcgaacccgagacatcagcttaaggacgaaggatttcttaccacttcaccacaacctttatacccaaacataatctagtaacttggtttattgtctcatgatattatccaaagactaaaagacaatcaaaagaaagttcaaaagttgtggcagcatgataaagaattacacttactgagatgatggttgcatcaattaatgtatgaacatgatggtatcaaataccaatcattgaatattatattatttggatgcttgcatttttcaacatgcttttgtccttttggatatagtctaattttgagctcagt

SEQ ID NO: 6 - DNA, 7160 bp, Nicotiana tabacum
  source 1..7160: mol_type = genomic DNA
atagttgtccatgacgttttcagtttaatccttcacccaatccaacaaactaatgtttaatagtggtttctaaatcgagttaaggtattcatgaaattttgcaagtttttgaaaattttttgaaaatgagtttttcaaaaatcaaaaagtgattttgaccactttttcataattttcataaaattattttccactaacaaaattgcaatattttttcaagtgaaatgcatgtctaaacataatttctaactccaaatactatttttttttttttttttttttttttttcnnnnnnnnnnnnnnnnnnnnnnnnnnnnnnnnnnnnnnnnnnnnnnnnnnnnnnnnnnnnnnnnnnnnnnnnnnnnnnnnnnnnnnnnnnnnnnnnnnnnnnnnnnnnnnnnnnnnnnnnnnnnnnnnnnnnnnnnnnnnnnnnnnnnnnnnnnnnnnnnnnnnnnnnnnnnnnnnnnnnnnnnnnnnnnnnnnnnnnnnnnnnnnnnnnnnnnnnnnnnnnnnnnnnnnnnnnnnnnnnnnnnnnnnnnnnnnnnnnntgtccaaacgcctactagatgtgttacaaaatgatatttgggctattttgatagataaattattttggactagttggtgaaaattatttatggactgaccttcaaaaaaagcttctcaacattttcagaacgaaataactccagcaaatcaaatctatccacgtgtcatttttgagaaatgacaataacacatcagcaaaaagcttccctccttcctatccataacttcgctctctgtccatccaaaaaaccagcaaagactcacaaaactccattctgatttcagcttcaattcttgctaatttttcatgcattttcaattttcaaaaccccattaaaccaaaagaatgaatgaaaatctcatattttgaaaaatctcgagaaaagaaaaataaaaacagagaagtcagataaagaatatatatttacattgagataatatatactcaaaaatggattgtattggagctcgaaattttgctacaatggcggtttttacgtgtccgagattcaaatcattaggaagaaggagaattatgccaagaaaaaagcaaccaatttggcctatacatatgcaagtgaagtgtagtggaaatgagagttgtgtagtagttaaagaagattttgccgatgaagaggattatataaaagctggtggttcagaacttgtttttgttcaaatgcagcagaataaagacatggatctgcagtctaagctttctgataaggtgattttcttgatcccatttttaataagtataaaagatattttacattatcagtgtagtttaatacagtgacggaagcagtattttcaccgaaaagtttcaagaaatagaaaaagaatatatatacacactgataatgtaattcttcgcgaaatgggttcggctgaacccctcccgcccacctagctccgcccctagtttaagatgtgatagtaggtaaactctttactaggttataaattaatgtttatcatacatatttgcatgtaattaatttataagtaacctgattgtgtaagtatgcattgacaaggtaacaaattttacatttttagtggattttaaaattgttgtagcacgttacgtgtcttattttccaggtcgctaattccacttattatggatggttactatagttatctcttaggcacgagttgatagtatagagattcttttagcctatcagtgtttatataagttaaactctttaaaaagggattaacatatatactgactgtgtaaaaaatgtttagatcctcttgttattattgtttgttgctaatgcttcctttcacctttcttgaaccaatgatctatcgaaagtagcctctctaccttcaccaggtaggggtaaggtctgcgtacacacttccctccctagaccctatttgtgggattacaccgggtttgttgttgtagtaaaaaatgtttagactattgtgtagtttaataagcttatagtgtaggaatctttttgtagttttagtcggcgtttggacataagaattgtaaaattccaaaatagggggaaaattttttcaagcgaaaatggtatttgaaatttagagttgtatttggacatgaatataattttgggttgtttttgaagttttgtgaatgatttgtgtgaaaattttgaaaaataactttttggagtttttcaaatttttgaaaattttcaaaatgcatcttcgagtgaaaattggaaattttatgaacaaacgctcatttcaaaaaaaaagtgaaatgtttttggaaaaaaggaaaaattttcttatgtccaaacgggctcttaatactatttaaccggttgtaatatgttacttacctatattaccatctcccacatagtattgaaagcaatatgtagttagcttgggaaaatatttacaatgttagtgtaaattctgtaatatggtagcaactacattgctttggtctctaatactgtagcaactattagttctcatatctagcaactatattgctttgttcatcatactatctcagcttgcagttgcgacaaatatcatcagctggacaaactatactggatttggtggtcataggctgtggtcctgctggtcttgctcttgctgcggagtctgctaaactcggattgaacgttgggctcgttggtcctgatcttcctttcacaaataactatggtgtttgggaggatgagttcaaaggtcgtaatctttatttggcttttatcaagaactagtttgtctccctatcctttcaagaaacaggacactttgttttactttcttgaaacaattagctaaaaagcacattgtatttccttttatcaaatgctagattcataggacttgttacattcacccttttagcaatttgtcaacttgagatccaagagatagttaatttcacagacataaactgatacttgaagtaatcactttactttagttatatgcatgagcaccggcaacaacaacaacatcgtgtaatctcataagtgggttctggggaaggtagtgagtacgtaaccttactcctacattgtgcaggtaaatagactgtttccgatagatatatgcatgagcactggatctgtcattattggttttgaggtttttgatactcaacttggtttttcactgcaaaattgatgtttaggatatgatattccaggctaaaattactctccaaacttcatatgcttaatactttcttttttcagatcttgggcttcaagcgtgcattgaacatgtttggagggataccatagtatatcttgacgatgccgatccaattcttatcggtcgtgcttatggaagagttagtcgccatttactgcacgaggagttactcaaaaggttaaattcactgaacttgttccttatgtaatacaagttgttaatttattcttttcaattgtttcatcattttattttccttaaaagttgcaattcacattaatcttcttaggtgtgtggaggcaggtgttttatatcttaactcgaaagtggataggatcgttgagtccacaagtggccacagtcttgtagagtgcgagggcgacattgtcattccttgcaggtatagttggaccgctacttcaaattgtcgctgttcacgttagaaacttaactgcatccttgttctgacgcttctaacttatgataacaggtttgtcactgttgcatctggtgctgcctcagggaaattcttgcagtatgagttgggaggtcctcgggtttctgttcaaacagcttatggagtggaagttgaggtagagaaagatcatcaaacataagtaactctgaagttttttcatgttatacactcgaagaacattaaactgttatctctagctatcgtttacgagcttatatgaacaaattgttgcattattcctttttttggcttatccttacactgctcgtctcggagaatatgtattcaatttgacgattctgtttctattgtaaacgtagaatgggacttcctattcatcagataaaaggaaactactataatgttatgcacattcaagaaactgctatctgcatttcccaattatcagttatggcacctaacttggctaattctgcaattatatgatcattcttcttcttttttccctatatattaggtcgataacaatccgtatgatccaagcctgatggttttcatggattatagagactatgtcagacacgacgctcaatctttagaagctaaatatccaacatttctttatgccatgcccatgactaaaacaagagtctttttcgaggttagtttttgatattatgcctcacactttacgacttggctatatgtgacagataaaagtatctatctgtaggaaacttgtttggcttcaaaagatgcaatgccatttgatttgttaaagaaaaaactgatgttacgattgaacacactgggtgtaagaattaagcaaatctacgaggaggtaatccactctgcctttagttacgtgcaatttttgctagagaaaaaagggatgcccagtgtattaagcacccgctatgcgcggggtgtggggaagggccagatcacaagggtctattgcacgcaaccttaccctgcatttctgcaagagactatttccacggctcgaaccccgtgacttcctggtcgcatggcaacaactttaccagttatgccaagactccccgtgaacacactagagaatgactgaaaaatgacgataacaaaattttacgcaggaatggtcatacataccagttggtggatctttaccaaataccgagcaaaaaacacttgcatttggtgctgctgctagcatggttcatccagctacaggtaataagagaagaaaatacattactattactgtgttctttaaatgcaatgcttctgaaacttcctctactgcattaacaggttattcagttgtcagatcactgtccgaggcaccaaaatgcgcctccgtacttgctaatattttacgacaaaatcatgtcaagaacatgctaaccagttcaagtaccacaagtatctcaactcaaggtacttgttatccaattatactagtttttgactgcatttgtagtgtcctgacctttatagactcagcaagttgctcatattttcttcagcttggaacaccctttggccacaagaacgaaaaaggcaacgatcgtttttcctatttggattggcactcatattgcagttggatattgaggggattaggtcatttttccgcgcattcttccgtgtgccaaaatggtatggtttgatcttgctccatcaccccgttatcttcgatgatgtagcatcgtattccaaatcaatttaacttctatacacttacaatataaataatatttatactacaagatgatcaaaaaacaaataagtacatgtaactgtttataataagtgaaattaataatgcacaaaataaggcagttcaacatgatacaacaggttaagaacattaataccaacaacaacaacaacaactatgccctcagtaccaaacaagttggagcggctatcaggggcggagctagagtgccccgagcaggttctgccgaacccaatagttttggttcgaaccctctatttgtcttaaaaaattcattgaatatatataaattattaatttacaacctaataccttaaaacgagtagaattccgaacccataaacttgaaatcttggctccgcctctggcagctatatgaatcctcaatgaccatattccctatttaaattcttctcaagtcaacattatacgaaacaaaaatcaaaacgaaaagtacgtacaagttttctatgtttccaactgacataagaatcccaaaagcgtaaatttcttaaactgtcagtgtatataagttaagtccttcccgaatacaaaaagaaacttctagtttcaacagtactaatgaggagtgtacttattgcaggatgtggcaaggatttcttggctctagtctttcatcagcagacctcatgttatttgccttctacatgtttattattgcaccaaatgacatgagaaaaggcctaatcagacatttgttatctgatccaactggtgcaaccatgataagaacttatcttacattttagagtagttccttctacattagttcttgaatctgttctctagaacagatgcctcatcatttcagattcataatagaatccgccgcctctcgaggctttgtatataacatcttgactaggttaatatggttaaataaattagccaatttcattttgtatctgcttctttgtccagatgtaatgattcattgcactctattagcttcaataaatggctgttagagagaacacacttctatttacttaattatgccttcaacacccccctatgtgtgggtttgatctttttgatgagccaagtacgtggaaattgtttctgatattggttggcggtgagattcgaacccaggacctttgcctgctctgataccatgttgaagtatgtgaccatatcatttaaaagcttaaactgttagcatatttttttttgcttaattatatatttaacatgtatacgagaaagacgcgttatagacttataatgaaataaatcaatctttgagataaggctcaaatgtttgtgttggggtaggctgtctacatcacacccttcgggatacagctctttcccggatcatgcatgaacgcgggatgctttgtgcactaggatgccctttttgtctttttcagatgagacgtttcatattattattatttaatatagaagagcttttgcctataactataacgtccctactttgactagtacccaaacatatctagcaactcgagtacttgtctcacgatataatccaaagacagagacaatcaaaagaaagtttaagcccccgtttggctatagatttggtaggtggttatgaaaaacaattgaaaacaatatttgttcatagaatatgatcagtttttgagaattttttttttaaattctcaaaagctggttttcggcagtgtttgggtgaaaattttcttccaacacacaacatcacaacttttttttcaaataaaatgcatgtccaaatacaatttcaacttccaaaaatta

SEQ ID NO: 7 - DNA, 19 bp, synthetic construct
  misc_feature 1..19: note = Synthetic primer
  source 1..19: mol_type = other DNA
aagtgatagttgtgtagtg

SEQ ID NO: 8 - DNA, 19 bp, synthetic construct
  misc_feature 1..19: note = Synthetic primer
  source 1..19: mol_type = other DNA
ctgatcctgacataacttg

SEQ ID NO: 9 - DNA, 19 bp, synthetic construct
  misc_feature 1..19: note = Synthetic primer
  source 1..19: mol_type = other DNA
actggatttagtggtcatt

SEQ ID NO: 10 - DNA, 19 bp, synthetic construct
  misc_feature 1..19: note = Synthetic primer
  source 1..19: mol_type = other DNA
aagctccagagaacaagag

SEQ ID NO: 11 - DNA, 18 bp, synthetic construct
  misc_feature 1..18: note = Synthetic primer
  source 1..18: mol_type = other DNA
aaaacagagaagtcagat

SEQ ID NO: 12 - DNA, 18 bp, synthetic construct
  misc_feature 1..18: note = Synthetic primer
  source 1..18: mol_type = other DNA
cttcacttgcatatgtat

SEQ ID NO: 13 - DNA, 19 bp, synthetic construct
  source 1..19: mol_type = other DNA
aagtgtagtggaaatgaga

SEQ ID NO: 14 - DNA, 19 bp, synthetic construct
  source 1..19: mol_type = other DNA
aatactgcttccgtcactg